European Patent Specification EP 3 653 707 B1, published July 16, 2025. Title: COMPOSITIONS AND METHODS COMPRISING LG12-CLADE PROTEASE VARIANTS. Applicant: DANISCO US INC. Application PCT/US14/55223. The sequence listing filed with the application follows.

SEQUENCE LISTING (29 sequences)

SEQ ID NO: 1 - DNA, 1143 bp, Artificial Sequence
  Synthetic: nucleotide sequence encoding the precursor to LG12 sprC protein as encoded in plasmid pHYT-LG12
gtgagaagcaaaaaattgtggatcagtttgctgtttgctttagcgttaatctttacgatggcgttcggcagcacatcctctgcccaggcggcagggaaatcaaacggggaaaagaaatacttagttggatttgcaaaaggtaataaagcaaatgcccagtcttctaaaaatttgattactgctgctggtggggacatacaacatacattccagtacatggatgttgtggaagtatcattgcctgaaaaagctgcagaagcattaatgaagaatcctaacattgctttcgttgaggaaaacgtcgaaatgatggctactgctcaaacagttccttggggcatccctcatatcaaagctgacaaagcgcatgctgctggagtgactggaagcggtgtgaaggttgccatcctggatacaggaattgacgcaaaccatgccgatcttaacgtaaaaggcggagcaagctttgtttctggagagccgaatgctcttcaagacggtaacggccatggaacacacgtagctggaacagttgctgcgttgaataacacaactggtgtacttggtgtagcttacaatgctgacctgtatgcagtaaaagtacttagtgcttcaggtagtggtacgttaagtggtattgctcaaggtattgagtggtcgatctcaaatggaatgaatgtcatcaatatgagtcttggtggaagctctggttcaactgctttacaacaagcgtgtaataatgcttataacagaggcattgtcgtaattgctgctgctgggaattcaggttcttcaggcaatcggaatacgatgggttatcctgcgagatatagctctgtaatcgcagtaggagcggttagtagcaataatactcgtgcatcattctccagtgtaggaagtgaactggaagtaatggcaccaggtgtcaacattttgagcacaactcctggcaacaattatgcttccttcaatggtacatccatggcagctcctcatgttgcaggagctgctgcattaatcaaagcgaaatacccaagcatgacaaatgttcaaattcgtgaacgtctgaaaaatacggctacaaatctaggtgatcctttcttctacggaaaaggtgtcatcaatgtggaaagtgctttacag

SEQ ID NO: 2 - DNA, 825 bp, Bacillus sp. Strain LG12
  misc_feature (1)..(825): nucleotide sequence coding for mature LG12 sprC protein
gctcaaacagttccttggggcatccctcatatcaaagctgacaaagcgcatgctgctggagtgactggaagcggtgtgaaggttgccatcctggatacaggaattgacgcaaaccatgccgatcttaacgtaaaaggcggagcaagctttgtttctggagagccgaatgctcttcaagacggtaacggccatggaacacacgtagctggaacagttgctgcgttgaataacacaactggtgtacttggtgtagcttacaatgctgacctgtatgcagtaaaagtacttagtgcttcaggtagtggtacgttaagtggtattgctcaaggtattgagtggtcgatctcaaatggaatgaatgtcatcaatatgagtcttggtggaagctctggttcaactgctttacaacaagcgtgtaataatgcttataacagaggcattgtcgtaattgctgctgctgggaattcaggttcttcaggcaatcggaatacgatgggttatcctgcgagatatagctctgtaatcgcagtaggagcggttagtagcaataatactcgtgcatcattctccagtgtaggaagtgaactggaagtaatggcaccaggtgtcaacattttgagcacaactcctggcaacaattatgcttccttcaatggtacatccatggcagctcctcatgttgcaggagctgctgcattaatcaaagcgaaatacccaagcatgacaaatgttcaaattcgtgaacgtctgaaaaatacggctacaaatctaggtgatcctttcttctacggaaaaggtgtcatcaatgtggaaagtgctttacag

SEQ ID NO: 3 - protein, 275 aa, Bacillus sp. Strain LG12
  misc_feature (1)..(275): amino acid sequence of the mature LG12 sprC protein
AQTVPWGIPHIKADKAHAAGVTGSGVKVAILDTGIDANHADLNVKGGASFVSGEPNALQDGNGHGTHVAGTVAALNNTTGVLGVAYNADLYAVKVLSASGSGTLSGIAQGIEWSISNGMNVINMSLGGSSGSTALQQACNNAYNRGIVVIAAAGNSGSSGNRNTMGYPARYSSVIAVGAVSSNNTRASFSSVGSELEVMAPGVNILSTTPGNNYASFNGTSMAAPHVAGAAALIKAKYPSMTNVQIRERLKNTATNLGDPFFYGKGVINVESALQ

SEQ ID NO: 4 - protein, 381 aa, Bacillus sp. Strain LG12
  misc_feature (1)..(381): amino acid sequence of the full-length LG12 sprC protein
VRSKKLWISLLFALALIFTMAFGSTSSAQAAGKSNGEKKYLVGFAKGNKANAQSSKNLITAAGGDIQHTFQYMDVVEVSLPEKAAEALMKNPNIAFVEENVEMMATAQTVPWGIPHIKADKAHAAGVTGSGVKVAILDTGIDANHADLNVKGGASFVSGEPNALQDGNGHGTHVAGTVAALNNTTGVLGVAYNADLYAVKVLSASGSGTLSGIAQGIEWSISNGMNVINMSLGGSSGSTALQQACNNAYNRGIVVIAAAGNSGSSGNRNTMGYPARYSSVIAVGAVSSNNTRASFSSVGSELEVMAPGVNILSTTPGNNYASFNGTSMAAPHVAGAAALIKAKYPSMTNVQIRERLKNTATNLGDPFFYGKGVINVESALQ

SEQ ID NO: 5 - DNA, 1080 bp, Bacillus sp. m3-13
  misc_feature (1)..(1080): nucleotide sequence encoding the precursor to Bacillus sp. m3-13 subtilisin E(1) protein used for cloning gene into pHYT vector using NheI-HindIII sites
gctagcgcagcagcttctggtccgagtgctaatgccaagaaagagtacttagtgggatttgctaaaggaaacaaagcgaatgctcagtcttccaaaaatttaattacagctgctggtggcgatattcaacatacattccagtacatggatgtagtggaagtgagcttgcctgaaaaagcggctgaagcattagcgaaaaatcctaacattgcatttgtagaggtaaacgcagaagttcaagctactgcacaaacagttccttggggaattcctcacattaaagcagacaaagcgcacgcttcaggtgtaacaggaagtggagtgaaagttgcggtccttgatacaggaattgatgcaaaccatgcggatttgaatgttaaaggtggagcaagctttgtttctggtgaaccaaatgcccttcaagatggaaacgggcacggaacacacgtagcaggaacggttgctgcattgaataatacgacaggagtgcttggtgtagcttataatgcggatctttatgcagttaaagttcttagtgcttccggaagcggtacattaagtggaatcgcacaaggaattgagtggtccattgctaatgatatggacgttatcaatatgagccttggtggtagtaccggttccacagcacttcagcaagcttgtgacaatgcatatgcaagtggaattgtagtggttgcagctgctggaaactccggttctaaaggtaagagaaacacaatgggttaccctgctagatacagttctgtaattgcagttggtgcggtcgacagcagtaacaaccgtgcatctttctcaagtgttggaagtgagcttgaagtaatggctccaggtgtaagtatccttagcacgactcctggaaacaactactcttccttcaatggtacgtctatggcttctccacatgttgcaggagcagctgcattaatcaaagcaaaatatcctagcatgacgaatgtacaaattcgtgaaaaactaaaaaatactgccactaaccttggcgatgcgttctattatggacatggtgtaattaacgttgaaagtgctttgcaataaaagctt

SEQ ID NO: 6 - protein, 383 aa, Bacillus sp. m3-13
  misc_feature (1)..(383): amino acid sequence of the full length Bacillus sp. m3-13 subtilisin E(1) protein as expressed from gene sequence SEQ ID NO:5 in pHYT plasmid
MRSKKLWISLLFALTLIFTMAFSNMSASAAASGPSANAKKEYLVGFAKGNKANAQSSKNLITAAGGDIQHTFQYMDVVEVSLPEKAAEALAKNPNIAFVEVNAEVQATAQTVPWGIPHIKADKAHASGVTGSGVKVAVLDTGIDANHADLNVKGGASFVSGEPNALQDGNGHGTHVAGTVAALNNTTGVLGVAYNADLYAVKVLSASGSGTLSGIAQGIEWSIANDMDVINMSLGGSTGSTALQQACDNAYASGIVVVAAAGNSGSKGKRNTMGYPARYSSVIAVGAVDSSNNRASFSSVGSELEVMAPGVSILSTTPGNNYSSFNGTSMASPHVAGAAALIKAKYPSMTNVQIREKLKNTATNLGDAFYYGHGVINVESALQ

SEQ ID NO: 7 - protein, 275 aa, Bacillus sp. m3-13
  misc_feature (1)..(275): amino acid sequence of the mature Bacillus sp. m3-13 subtilisin E(1) protein
AQTVPWGIPHIKADKAHASGVTGSGVKVAVLDTGIDANHADLNVKGGASFVSGEPNALQDGNGHGTHVAGTVAALNNTTGVLGVAYNADLYAVKVLSASGSGTLSGIAQGIEWSIANDMDVINMSLGGSTGSTALQQACDNAYASGIVVVAAAGNSGSKGKRNTMGYPARYSSVIAVGAVDSSNNRASFSSVGSELEVMAPGVSILSTTPGNNYSSFNGTSMASPHVAGAAALIKAKYPSMTNVQIREKLKNTATNLGDAFYYGHGVINVESALQ

SEQ ID NO: 8 - DNA, 1143 bp, Bacillus horikoshii strain DSM 8719
  misc_feature (1)..(1143): nucleotide sequence of the Bhon03321 gene
ttgaagaagtggatgaagagtttttcagttatacttattgcaatattggctttctcgttagcttttggaactgctcaggcagagtcttctaatccgaatgctagtgtaaagaaagaatacttaattgggtttgcaaaaggaaacaaggcaagtgcacagacctcccaaaatctggttacagcagcagggggagaagttcaacacacattccaatacatggatgtagtggaagtttcgttacctgaaaaagctgcagaagcattgaagaagaatcctaacatagcattcgtagaggaaaacgtagaggttatggcgactgcccaaacagtaccttggggcatcccgcatatcaaagcagacaaagcacatgctgccggtgtgacaggaagcggagtgaaagtggcaatccttgatacagggatcgacgccaatcatgcagacttaaatgtaagaggcggagcaagttttgtggcaggtgagccgaatgcccttcaagatggaaatggacacggaactcacgtggccggtacggttgccgcattgaataattcaactggcgttctaggggtcgcttacaacgcagacctttatgcggtaaaagttcttagcgcttcaggtagtgggactttaagtggcatcgcacaaggtattgaatggtccattgcaaatggaatggatgtaatcaatatgagtcttggtggaagctctgggtctactgcactccaacaagcttgtaataatgcctacaatagaggcattgttgtaattgctgctgctgggaattccggctcttcaggaaatcgcaacactatcgggtaccctgcaagatatagttcagtaatcgcagtgggagcagtggattccaataacaaccgcgcttctttctccagtgttggaaatgagctggaagtaatggcgccgggtgctaatatcttgagcacgactcctggtaataactatgcatccttcaacggaacgtccatggcagctccacatgttgcaggagcagcagcattgataaaagcaaaatatcctagcatgacaaatgtccaaattcgtgatcgtttaagaaatacggctacaaaccttggtgatcctttcttttatggaaacggagtaatcaatgtagaaagtgctttacaa

SEQ ID NO: 9 - protein, 381 aa, Bacillus horikoshii strain DSM 8719
  misc_feature (1)..(381): amino acid sequence of the serine protease precursor Bhon03321
MKKWMKSFSVILIAILAFSLAFGTAQAESSNPNASVKKEYLIGFAKGNKASAQTSQNLVTAAGGEVQHTFQYMDVVEVSLPEKAAEALKKNPNIAFVEENVEVMATAQTVPWGIPHIKADKAHAAGVTGSGVKVAILDTGIDANHADLNVRGGASFVAGEPNALQDGNGHGTHVAGTVAALNNSTGVLGVAYNADLYAVKVLSASGSGTLSGIAQGIEWSIANGMDVINMSLGGSSGSTALQQACNNAYNRGIVVIAAAGNSGSSGNRNTIGYPARYSSVIAVGAVDSNNNRASFSSVGNELEVMAPGANILSTTPGNNYASFNGTSMAAPHVAGAAALIKAKYPSMTNVQIRDRLRNTATNLGDPFFYGNGVINVESALQ

SEQ ID NO: 10 - protein, 275 aa, Bacillus horikoshii strain DSM 8719
  misc_feature (1)..(275): amino acid sequence of the mature Bhon03321 protease
AQTVPWGIPHIKADKAHAAGVTGSGVKVAILDTGIDANHADLNVRGGASFVAGEPNALQDGNGHGTHVAGTVAALNNSTGVLGVAYNADLYAVKVLSASGSGTLSGIAQGIEWSIANGMDVINMSLGGSSGSTALQQACNNAYNRGIVVIAAAGNSGSSGNRNTIGYPARYSSVIAVGAVDSNNNRASFSSVGNELEVMAPGANILSTTPGNNYASFNGTSMAAPHVAGAAALIKAKYPSMTNVQIRDRLRNTATNLGDPFFYGNGVINVESALQ

SEQ ID NO: 11 - DNA, 1146 bp, Bacillus horikoshii DSM 9711
  misc_feature (1)..(1146): nucleotide sequence of the DSM9711_sprC gene
ttgaagaagtggatgaaaggtttttcggtcatacttattgcaatattggctttctcgttagcatttggtactgcgcaggcagaatcgtccagtcccaatgctagtgcaaagaaagaatacttagttggctttacaaaaggaaataaggcaagtgcacaatcttctaaaaacttgattgccgcagcaggtggggaagtacagcacacgttccaatacatggatgttgtggaagtgtctttacctgaaaaagcggtagatgcattgaagaaaaatcctaacatcgcttttgtagaagaaaacgcagaagttcaagcaactgcacaaactgtgccatggggtatccctcatatcaaggctgacaaagcgcatgcctctggtgtgacaggaagcggtgtcaaagtcgcgatcctagatacaggaattgacgcaaaccatactgatcttaatgtaaaaggcggagcgagctttgtttcaggtgagccaaatgcccttcaagatggtaacggccatggaacacacgtagcaggaacagttgctgcgttaaataattctactggtgtacttggtgtagcttacaatgctgacctttatgcggtgaaagtacttagtgcttcaggtagtggaacattaagtggaatcgcacaagggattgagtggtccattgcaaatggaatgaacgtcatcaatatgagtttaggaggcagcactggatcaactgcattgcaacaagcttgtgataatgcttatgcaagaggtattgtcgtcattgcggcagctggaaactctggttctagagggaagcaaaacacaatgggttatcctgcaagatacagctccgtcatcgcagtaggagcggtagattccagtaacaaccgtgcttctttctccagtgtaggaaacgaattggaagtaatggcaccgggtgttaacattttaagcacaactcctggtaacaactatgcatccttcaatggaacgtccatggcgtctccacacgttgctggagctgctgcattaatcaaagcgaagtatccaagcatgacaaatgttcaaatccgtgaccgtctgaaaaatacggctacaaacttaggtgatcctttcttctacggtaaaggtgtcatcaatgtggaaagtgctttacaataa

SEQ ID NO: 12 - protein, 381 aa, Bacillus horikoshii DSM 9711
  misc_feature (1)..(381): amino acid sequence of the serine protease precursor of DSM9711_SprC
MKKWMKGFSVILIAILAFSLAFGTAQAESSSPNASAKKEYLVGFTKGNKASAQSSKNLIAAAGGEVQHTFQYMDVVEVSLPEKAVDALKKNPNIAFVEENAEVQATAQTVPWGIPHIKADKAHASGVTGSGVKVAILDTGIDANHTDLNVKGGASFVSGEPNALQDGNGHGTHVAGTVAALNNSTGVLGVAYNADLYAVKVLSASGSGTLSGIAQGIEWSIANGMNVINMSLGGSTGSTALQQACDNAYARGIVVIAAAGNSGSRGKQNTMGYPARYSSVIAVGAVDSSNNRASFSSVGNELEVMAPGVNILSTTPGNNYASFNGTSMASPHVAGAAALIKAKYPSMTNVQIRDRLKNTATNLGDPFFYGKGVINVESALQ

SEQ ID NO: 13 - protein, 275 aa, Bacillus horikoshii DSM 9711
  misc_feature (1)..(275): amino acid sequence of the mature protease DSM9711_SprC
AQTVPWGIPHIKADKAHASGVTGSGVKVAILDTGIDANHTDLNVKGGASFVSGEPNALQDGNGHGTHVAGTVAALNNSTGVLGVAYNADLYAVKVLSASGSGTLSGIAQGIEWSIANGMNVINMSLGGSTGSTALQQACDNAYARGIVVIAAAGNSGSRGKQNTMGYPARYSSVIAVGAVDSSNNRASFSSVGNELEVMAPGVNILSTTPGNNYASFNGTSMASPHVAGAAALIKAKYPSMTNVQIRDRLKNTATNLGDPFFYGKGVINVESALQ

SEQ ID NO: 14 - DNA, 1152 bp, Bacillus horikoshii DSM 9712
  misc_feature (1)..(1152): nucleotide sequence of the DSM9712_sprC  gene
ttgaagaagtggatgaaaggtttttcggtcatacttatagcaatattggctttctcattagccttcggaactggaactgcccaggcggaatcttcaggaccgagtgctggtgcaaagaaagagtacttaattggatttacgaaaggaaataaagcaagcgcacaatcctcccaaaatctagtcactgctgcaggtggcgatattcaatacacattccaatacatggatgtagtggaagtaactttacctgaaaaagctgctgaggcattaaagaagaaccctaacattgcatttgtagaggaaaacgtagaaatgatggcgactgcacagacagtaccatggggtattccgcacatcaaagcagataaggcacatgccgctggtgtaactggaagtggtgtgaaggtagcgatccttgacacaggaattgacgctaaccatgccgaccttaatgtaaaaggtggagcaagctttgtttctggtgaaccaaatgccctacaagatggcaatggccatggaacacatgtagcgggaacggttgctgcgttaaataacacaactggtgtgcttggagtggcttacaatgcggatctttatgcagttaaagtccttaacgcatctggtagtgggacgttaagtggcattgcccaaggaattgagtggtccattgcaaatggaatggatgtaatcaatatgagccttggtggcagcactggatcaactgcattacaacaagctagtaataatgcttacaatagaggcattgtcgtcattgcagctgccggaaattcaggttctttaggcaatcggaatacaattgggtatcctgccagatatagttctgttatcgcggtaggagcggttgactccaacaacaaccgtgcttccttctctagtgtaggaagtgaattggaagtaatggcacctggtgtaaatattctgagcacgactcctggtaataactatgcttctttcaatggtacatctatggcagctccacatgttgcaggagcagcagcattaatcaaggcgaaatacccgaatatgacaaacgtccaaattcgtgatcgcctgagaaatacagctacaaaccttggtgatccattcttctatggaagaggagtcatcaatgtggaaagtgctttacaataa

SEQ ID NO: 15 - protein, 383 aa, Bacillus horikoshii DSM 9712
  misc_feature (1)..(383): amino acid sequence of the serine protease precursor of DSM9712_SprC
MKKWMKGFSVILIAILAFSLAFGTGTAQAESSGPSAGAKKEYLIGFTKGNKASAQSSQNLVTAAGGDIQYTFQYMDVVEVTLPEKAAEALKKNPNIAFVEENVEMMATAQTVPWGIPHIKADKAHAAGVTGSGVKVAILDTGIDANHADLNVKGGASFVSGEPNALQDGNGHGTHVAGTVAALNNTTGVLGVAYNADLYAVKVLNASGSGTLSGIAQGIEWSIANGMDVINMSLGGSTGSTALQQASNNAYNRGIVVIAAAGNSGSLGNRNTIGYPARYSSVIAVGAVDSNNNRASFSSVGSELEVMAPGVNILSTTPGNNYASFNGTSMAAPHVAGAAALIKAKYPNMTNVQIRDRLRNTATNLGDPFFYGRGVINVESALQ

SEQ ID NO: 16 - protein, 275 aa, Bacillus horikoshii DSM 9712
  misc_feature (1)..(275): amino acid sequence of the mature protease DSM9712_SprC
AQTVPWGIPHIKADKAHAAGVTGSGVKVAILDTGIDANHADLNVKGGASFVSGEPNALQDGNGHGTHVAGTVAALNNTTGVLGVAYNADLYAVKVLNASGSGTLSGIAQGIEWSIANGMDVINMSLGGSTGSTALQQASNNAYNRGIVVIAAAGNSGSLGNRNTIGYPARYSSVIAVGAVDSNNNRASFSSVGSELEVMAPGVNILSTTPGNNYASFNGTSMAAPHVAGAAALIKAKYPNMTNVQIRDRLRNTATNLGDPFFYGRGVINVESALQ

SEQ ID NO: 17 - DNA, 1146 bp, Bacillus horikoshii DSM 6951
  misc_feature (1)..(1146): nucleotide sequence of the DSM6951_sprC gene
ttgaaaaagtggatgaaaggtttttcggtcatacttatcgcaatattggctttctcgttagccttcggaactgctcaggcagaagcatcaaatccgaatgctagtgcaaagaaagaatacttagttggatttgcaaaaggtaataaagcaaatgcccagtcttctaaaaatttgattaccgctgctggtggggacatacaacatacattccagtacatggatgttgtggaagtatcgttgcctgtaaaagctgcagaagcattaatgaagaatcctaacattgctttcgttgaggaaaacgtcgaaatgatggctactgctcaaacagttccttggggcatccctcatatcaaagctgacaaagcgcatgctgctggagtgactggaagcggtgtgaaggttgccatcctggatacaggaattgacgcaaaccatgccgatcttaacgtaaaaggcggagcaagctttgtttctggtgagccgaatgctcttcaagacggtaacggccatggaacacacgtagctggaacagttgctgctttgaataacacaactggtgtacttggtgtagcttacaatgctgacctatatgcagtaaaagtacttagtgcttcaggtagtggaacattaagtggcattgcgcaaggtattgagtggtccgttgctaacggaatggatgtcatcaatatgagtcttggtggaagctctggatcttcagctttacaacaagcttgtgataatgcttatgctagaggagttgtagtaattgccgcagctgggaactctggttcaagaggaaagcaaaacacaatggggtatcctgctagatacagttctgttatcgcagtaggagcggtggattccagtaacaaccgtgcctctttctccagtgttgggaatgaactggaagtaatggctcctggagtgaatattttaagcacgactcctggtaataactatgcttctttcaatggtacgtccatggcatctccgcacgttgcaggagctgctgcattaatcaaggcgaaatacccaagcatgacaaatgttcaaattcgtgaacgtctgaaaaatacggctacaaatttaggtgatcctttcttctacggaaaaggtgtcatcaatgtggaaagtgctttacaataa

SEQ ID NO: 18 - protein, 381 aa, Bacillus horikoshii DSM 6951
  misc_feature (1)..(381): amino acid sequence of the serine protease precursor of DSM6951_SprC
MKKWMKGFSVILIAILAFSLAFGTAQAEASNPNASAKKEYLVGFAKGNKANAQSSKNLITAAGGDIQHTFQYMDVVEVSLPVKAAEALMKNPNIAFVEENVEMMATAQTVPWGIPHIKADKAHAAGVTGSGVKVAILDTGIDANHADLNVKGGASFVSGEPNALQDGNGHGTHVAGTVAALNNTTGVLGVAYNADLYAVKVLSASGSGTLSGIAQGIEWSVANGMDVINMSLGGSSGSSALQQACDNAYARGVVVIAAAGNSGSRGKQNTMGYPARYSSVIAVGAVDSSNNRASFSSVGNELEVMAPGVNILSTTPGNNYASFNGTSMASPHVAGAAALIKAKYPSMTNVQIRERLKNTATNLGDPFFYGKGVINVESALQ

SEQ ID NO: 19 - protein, 275 aa, Bacillus horikoshii DSM 6951
  misc_feature (1)..(275): amino acid sequence of the mature protease DSM6951_SprC
AQTVPWGIPHIKADKAHAAGVTGSGVKVAILDTGIDANHADLNVKGGASFVSGEPNALQDGNGHGTHVAGTVAALNNTTGVLGVAYNADLYAVKVLSASGSGTLSGIAQGIEWSVANGMDVINMSLGGSSGSSALQQACDNAYARGVVVIAAAGNSGSRGKQNTMGYPARYSSVIAVGAVDSSNNRASFSSVGNELEVMAPGVNILSTTPGNNYASFNGTSMASPHVAGAAALIKAKYPSMTNVQIRERLKNTATNLGDPFFYGKGVINVESALQ

SEQ ID NO: 20 - protein, 276 aa, Bacillus sp. KSM-LD1
  misc_feature (1)..(276): amino acid sequence of the mature protease sp. KSM-LD1, SB (BAD21128)
SQTVPYGVPHIKADVAHSQNVTGNGVKVAILDTGIDAAHEDLRVVGGASFVAGEPNALQDGNGHGTHVAGTVAALNNQVGVLGVAYDVDLYAVKVLGADGSGTLSGIAQGIEWSIANNMDVINMSLGGSTGSTTLKQAADNAYNSGLVVVAAAGNSGDFFGLINTIGYPARYDSVIAVGAVDSNNRRASFSSVGSQLEVMAPGVNILSTLPGNSYGSLNGTSMASPHVAGAAALLLAQDPTLTNVQVREILRDTATNLGSSFYYGNGVIDVEKALQ

SEQ ID NO: 21 - DNA, 93 bp, Artificial Sequence
  Synthetic
ggttaccttgaatgtatataaacattctcaaagggatttctaataaaaaacgctcggttgccgccgggcgttttttatgcatcgatggaattc

SEQ ID NO: 22 - DNA, 21 bp, Artificial Sequence
  Synthetic
ggatcctgactgcctgagctt

SEQ ID NO: 23 - protein, 275 aa, Bacillus sp.
  misc_feature (1)..(275): Bacillus_sp_BAD11988
AQTTPWGVTHINAHRAHSSGVTGSGVKVAILDTGIHASHPDLNVRGGASFISGESNPYIDSNGHGTHVAGTVAALNNTVGVLGVAYNAELYAVKVLSASGSGTLSGIAQGVEWSIANKMDVINMSLGGSSGSTALQRAVDNAYRNNIVVVAAAGNSGAQGNRNTIGYPARYSSVIAVGAVDSNNNRASFSSVGSELEVMAPGVSILSTVPGSSYASYNGTSMASPHVAGAAALLKAKYPNWSAAQIRNKLNSTTTYLGSSFYYGNGVINVERALQ

SEQ ID NO: 24 - protein, 276 aa, Bacillus sp.
  misc_feature (1)..(276): B_sp_sprD_AAC43581
AQTVPYGVPHIKADVAHAQNVTGSGVKVAVLDTGIDASHEDLRVVGGASFVSEEPDALTDGNGHGTHVAGTIAALNNNVGVLGVSYDVDLYAVKVLSAGGSGTLAGIAQGIEWAIDNNMDVINMSLGGSTGSTTLKQASDNAYNSGIVVIAAAGNSGSVLGLVNTIGYPARYDSVIAVGAVDSNNNRASFSSVGSQLEVMAPGVAINSTLPGNQYGELNGTSMASPHVAGAAALLLAQNPNLTNVQVRERLRDTATNLGSAFNYGHGVINLERALQ

SEQ ID NO: 25 - protein, 276 aa, Bacillus sp.
  misc_feature (1)..(276): Bacillus_sp_WP_010192405
AQTVPYGVPHIKADVAHAQGVTGSGVKVAVLDTGIDASHEDLNVVGGASFVSEEPDALTDGNGHGTHVAGTIAAVNNNTGVLGVAYDVDLYAVKVLSAGGSGTLAGIAQGIEWAIDNDMDVINMSLGGSTGSSTLKQASDNAYNSGIVVVAAAGNSGSFFGLINTIGYPARYDSVIAVGAVDSNNNRASFSSVGSQLEVLAPGVSINSTLPGNQYGELNGTSMASPHVAGAAALLLAQNPNLTNVEVRERLRSTATNLGSSFNYGYGVINLEAALQ

SEQ ID NO: 26 - protein, 269 aa, Bacillus sp.
  misc_feature (1)..(269): B_lentus_P29600
AQSVPWGISRVQAPAAHNRGLTGSGVKVAVLDTGISTHPDLNIRGGASFVPGEPSTQDGNGHGTHVAGTIAALNNSIGVLGVAPSAELYAVKVLGASGSGSVSSIAQGLEWAGNNGMHVANLSLGSPSPSATLEQAVNSATSRGVLVVAASGNSGAGSISYPARYANAMAVGATDQNNNRASFSQYGAGLDIVAPGVNVQSTYPGSTYASLNGTSMATPHVAGAAALVKQKNPSWSNVQIRNHLKNTATSLGSTNLYGSGLVNAEAATR

SEQ ID NO: 27 - protein, 268 aa, Artificial Sequence
  Synthetic: consensus sequence
AQTVPWGIPHIKADKAHAAGVTGSGVKVAILDTGIDANHDLNVKGGASFVSGEPNALQDGNGHGTHVAGTVAALNNTTGVLGVAYNADLYAVKVLSASGSGTLSGIAQGIEWSIANGMDVINMSLGGSTGSTALQQADNAYNRGIVVIAAAGNSGSGNTIGYPARYSSVIAVGAVDSNNNRASFSSVGSELEVMAPGVNILSTTPGNNYASFNGTSMASPHVAGAAALIKAKYPSMTNVQIRERLKNTATNLGDFFYGGVINVESALQ

SEQ ID NO: 28 - protein, 275 aa, B. amyloliquefaciens [sequence omitted]

SEQ ID NO: 29 - protein, 274 aa, B. licheniformis
  misc_feature (1)..(274): carlsberg  - B_licheniformis_CAJ70731.1
AQTVPYGIPLIKADKVQAQGFKGANVKVAVLDTGIQASHPDLNVVGGASFVAGEAYNTDGNGHGTHVAGTVAALDNTTGVLGVAPSVSLYAVKVLNSSGSGSYSGIVSGIEWATTNGMDVINMSLGGASGSTAMKQAVDNAYARGVVVVAAAGNSGSSGNTNTIGYPAKYDSVIAVGAVDSNSNRASFSSVGAELEVMAPGAGVYSTYPTNTYATLNGTSMASPHVAGAAALILSKHPNLSASQVRNRLSSTATYLGSSFYYGKGLINVEAAAQ